European Patent Application EP 4 534 554 A1, published April 9, 2025. Title: MAGE-A1特异性TCR及其用途. Applicant: 北京可瑞生物科技有限公司. The sequence listing filed with the application follows.

SEQUENCE LISTING (177 sequences)

SEQ ID NO: 1 - protein, 594 aa, synthetic construct
  REGION 1..594: note = Full-length amino acid sequence of WT ht27 TCR
MLLLLLLLGPGSGLGAVVSQHPSWVICKSGTSVKIECRSLDFQATTMFWYRQFPKQSLMLMATSNEGSKATYEQGVEKDKFLINHASLTLSTLTVTSAHPEDSSFYICSAREPGQGPYEQYFGPGTRLTVTEDLRNVTPPKVSLFEPSKAEIANKQKATLVCLARGFFPDHVELSWWVNGKEVHSGVCTDPQAYKESNYSYCLSSRLRVSATFWHNPRNHFRCQVQFHGLSEEDKWPEGSPKPVTQNISAEAWGRADCGITSASYQQGVLSATILYEILLGKATLYAVLVSTLVVMAMVKRKNSSRATNFSLLKQAGDVEENPGPMKTFAGFSFLFLWLQLDCMSRGEDVEQSLFLSVREGDSSVINCTYTDSSSTYLYWYKQEPGAGLQLLTYIFSNMDMKQDQRLTVLLNKKDKHLSLRIADTQTGDSAIYFCAGSGGGTDKLIFGTGTRLQVFPNIQNPEPAVYQLKDPRSQDSTLCLFTDFDSQINVPKTMESGTFITDKCVLDMKAMDSKSNGAIAWSNQTSFTCQDIFKETNATYPSSDVPCDATLTEKSFETDMNLNFQNLLVIVLRILLLKVAGFNLLMTLRLWSS

SEQ ID NO: 2 - protein, 9 aa, synthetic construct
  REGION 1..9: note = MAGE-A1 epitope sequence
KVLEYVIKV

SEQ ID NO: 3 - protein, 306 aa, synthetic construct
  REGION 1..306: note = ht27M1001 b chain
MLLLLLLLGPGSGLGAVVSQHPSWVICKSGTSVKIECRSLDFQATTMFWYRQFPKQSLMLMATSDYQTCVTYEQGVEKDKFLINHASLTLSTLTVTSAHPEDSSFYICSAREPGQGPYEQYFGPGTRLTVTEDLRNVTPPKVSLFEPSKAEIANKQKATLVCLARGFFPDHVELSWWVNGKEVHSGVCTDPQAYKESNYSYCLSSRLRVSATFWHNPRNHFRCQVQFHGLSEEDKWPEGSPKPVTQNISAEAWGRADCGITSASYQQGVLSATILYEILLGKATLYAVLVSTLVVMAMVKRKNSSR

SEQ ID NO: 4 - protein, 306 aa, synthetic construct
  REGION 1..306: note = ht27M1002 b chain
MLLLLLLLGPGSGLGAVVSQHPSWVICKSGTSVKIECRSLDFQATTMFWYRQFPKQSLMLMATSNEGSKATYEQGVEKDKFLINHASLTLSTLTVTSAHPEDSSFYICSAREPGGGPYEQYFGPGTRLTVTEDLRNVTPPKVSLFEPSKAEIANKQKATLVCLARGFFPDHVELSWWVNGKEVHSGVCTDPQAYKESNYSYCLSSRLRVSATFWHNPRNHFRCQVQFHGLSEEDKWPEGSPKPVTQNISAEAWGRADCGITSASYQQGVLSATILYEILLGKATLYAVLVSTLVVMAMVKRKNSSR

SEQ ID NO: 5 - protein, 306 aa, synthetic construct
  REGION 1..306: note = ht27M1003 b chain
MLLLLLLLGPGSGLGAVVSQHPSWVICKSGTSVKIECRSLDFQATTMFWYRQFPKQSLMLMATSNEGSKATYEQGVEKDKFLINHASLTLSTLTVTSAHPEDSSFYICSAREPGSGPYEQYFGPGTRLTVTEDLRNVTPPKVSLFEPSKAEIANKQKATLVCLARGFFPDHVELSWWVNGKEVHSGVCTDPQAYKESNYSYCLSSRLRVSATFWHNPRNHFRCQVQFHGLSEEDKWPEGSPKPVTQNISAEAWGRADCGITSASYQQGVLSATILYEILLGKATLYAVLVSTLVVMAMVKRKNSSR

SEQ ID NO: 6 - protein, 306 aa, synthetic construct
  REGION 1..306: note = ht27M1004 b chain
MLLLLLLLGPGSGLGAVVSQHPSWVICKSGTSVKIECRSLDFQATTMFWYRQFPKQSLMLMATSNEGSKATYEQGVEKDKFLINHASLTLSTLTVTSAHPEDSSFYICSAREPGQGPFEQYFGPGTRLTVTEDLRNVTPPKVSLFEPSKAEIANKQKATLVCLARGFFPDHVELSWWVNGKEVHSGVCTDPQAYKESNYSYCLSSRLRVSATFWHNPRNHFRCQVQFHGLSEEDKWPEGSPKPVTQNISAEAWGRADCGITSASYQQGVLSATILYEILLGKATLYAVLVSTLVVMAMVKRKNSSR

SEQ ID NO: 7 - protein, 306 aa, synthetic construct
  REGION 1..306: note = ht27M1005 b chain
MLLLLLLLGPGSGLGAVVSQHPSWVICKSGTSVKIECRSLDFQATTMFWYRQFPKQSLMLMATSNEGSKATYEQGVEKDKFLINHASLTLSTLTVTSAHPEDSSFYICSAREPGQGPLEQYFGPGTRLTVTEDLRNVTPPKVSLFEPSKAEIANKQKATLVCLARGFFPDHVELSWWVNGKEVHSGVCTDPQAYKESNYSYCLSSRLRVSATFWHNPRNHFRCQVQFHGLSEEDKWPEGSPKPVTQNISAEAWGRADCGITSASYQQGVLSATILYEILLGKATLYAVLVSTLVVMAMVKRKNSSR

SEQ ID NO: 8 - protein, 306 aa, synthetic construct
  REGION 1..306: note = ht27M1006 b chain
MLLLLLLLGPGSGLGAVVSQHPSWVICKSGTSVKIECRSLDFQATTMFWYRQFPKQSLMLMATSNEGSKATYEQGVEKDKFLINHASLTLSTLTVTSAHPEDSSFYICSAREPGQGPWEQYFGPGTRLTVTEDLRNVTPPKVSLFEPSKAEIANKQKATLVCLARGFFPDHVELSWWVNGKEVHSGVCTDPQAYKESNYSYCLSSRLRVSATFWHNPRNHFRCQVQFHGLSEEDKWPEGSPKPVTQNISAEAWGRADCGITSASYQQGVLSATILYEILLGKATLYAVLVSTLVVMAMVKRKNSSR

SEQ ID NO: 9 - protein, 306 aa, synthetic construct
  REGION 1..306: note = ht27M1009 b chain
MLLLLLLLGPGSGLGAVVSQHPSWVICKSGTSVKIECRSLDFQATTMFWYRQFPKQSLMLMATSDYQTCVTYEQGVEKDKFLINHASLTLSTLTVTSAHPEDSSFYICSAREPGQGPFEQYFGPGTRLTVTEDLRNVTPPKVSLFEPSKAEIANKQKATLVCLARGFFPDHVELSWWVNGKEVHSGVCTDPQAYKESNYSYCLSSRLRVSATFWHNPRNHFRCQVQFHGLSEEDKWPEGSPKPVTQNISAEAWGRADCGITSASYQQGVLSATILYEILLGKATLYAVLVSTLVVMAMVKRKNSSR

SEQ ID NO: 10 - protein, 306 aa, synthetic construct
  REGION 1..306: note = ht27M1010 b chain
MLLLLLLLGPGSGLGAVVSQHPSWVICKSGTSVKIECRSLDFQATTMFWYRQFPKQSLMLMATSDYQTCVTYEQGVEKDKFLINHASLTLSTLTVTSAHPEDSSFYICSAREPGQGPLEQYFGPGTRLTVTEDLRNVTPPKVSLFEPSKAEIANKQKATLVCLARGFFPDHVELSWWVNGKEVHSGVCTDPQAYKESNYSYCLSSRLRVSATFWHNPRNHFRCQVQFHGLSEEDKWPEGSPKPVTQNISAEAWGRADCGITSASYQQGVLSATILYEILLGKATLYAVLVSTLVVMAMVKRKNSSR

SEQ ID NO: 11 - protein, 306 aa, synthetic construct
  REGION 1..306: note = ht27M1011 b chain
MLLLLLLLGPGSGLGAVVSQHPSWVICKSGTSVKIECRSLDFQATTMFWYRQFPKQSLMLMATSDYQTCVTYEQGVEKDKFLINHASLTLSTLTVTSAHPEDSSFYICSAREPGQGPWEQYFGPGTRLTVTEDLRNVTPPKVSLFEPSKAEIANKQKATLVCLARGFFPDHVELSWWVNGKEVHSGVCTDPQAYKESNYSYCLSSRLRVSATFWHNPRNHFRCQVQFHGLSEEDKWPEGSPKPVTQNISAEAWGRADCGITSASYQQGVLSATILYEILLGKATLYAVLVSTLVVMAMVKRKNSSR

SEQ ID NO: 12 - protein, 306 aa, synthetic construct
  REGION 1..306: note = ht27M1012 b chain
MLLLLLLLGPGSGLGAVVSQHPSWVICKSGTSVKIECRSLDFQATTMFWYRQFPKQSLMLMATSNEGSKATYEQGVEKDKFLINHASLTLSTLTVTSAHPEDSSFYICSAREPGGGPFEQYFGPGTRLTVTEDLRNVTPPKVSLFEPSKAEIANKQKATLVCLARGFFPDHVELSWWVNGKEVHSGVCTDPQAYKESNYSYCLSSRLRVSATFWHNPRNHFRCQVQFHGLSEEDKWPEGSPKPVTQNISAEAWGRADCGITSASYQQGVLSATILYEILLGKATLYAVLVSTLVVMAMVKRKNSSR

SEQ ID NO: 13 - protein, 306 aa, synthetic construct
  REGION 1..306: note = ht27M1013 b chain
MLLLLLLLGPGSGLGAVVSQHPSWVICKSGTSVKIECRSLDFQATTMFWYRQFPKQSLMLMATSNEGSKATYEQGVEKDKFLINHASLTLSTLTVTSAHPEDSSFYICSAREPGSGPFEQYFGPGTRLTVTEDLRNVTPPKVSLFEPSKAEIANKQKATLVCLARGFFPDHVELSWWVNGKEVHSGVCTDPQAYKESNYSYCLSSRLRVSATFWHNPRNHFRCQVQFHGLSEEDKWPEGSPKPVTQNISAEAWGRADCGITSASYQQGVLSATILYEILLGKATLYAVLVSTLVVMAMVKRKNSSR

SEQ ID NO: 14 - protein, 306 aa, synthetic construct
  REGION 1..306: note = ht27M1018 b chain
MLLLLLLLGPGSGLGAVVSQHPSWVICKSGTSVKIECRSLDFQATTMFWYRQFPKQSLMLMATSDYQTCVTYEQGVEKDKFLINHASLTLSTLTVTSAHPEDSSFYICSAREPGGGPFEQYFGPGTRLTVTEDLRNVTPPKVSLFEPSKAEIANKQKATLVCLARGFFPDHVELSWWVNGKEVHSGVCTDPQAYKESNYSYCLSSRLRVSATFWHNPRNHFRCQVQFHGLSEEDKWPEGSPKPVTQNISAEAWGRADCGITSASYQQGVLSATILYEILLGKATLYAVLVSTLVVMAMVKRKNSSR

SEQ ID NO: 15 - protein, 306 aa, synthetic construct
  REGION 1..306: note = ht27M1019 b chain
MLLLLLLLGPGSGLGAVVSQHPSWVICKSGTSVKIECRSLDFQATTMFWYRQFPKQSLMLMATSDYQTCVTYEQGVEKDKFLINHASLTLSTLTVTSAHPEDSSFYICSAREPGSGPFEQYFGPGTRLTVTEDLRNVTPPKVSLFEPSKAEIANKQKATLVCLARGFFPDHVELSWWVNGKEVHSGVCTDPQAYKESNYSYCLSSRLRVSATFWHNPRNHFRCQVQFHGLSEEDKWPEGSPKPVTQNISAEAWGRADCGITSASYQQGVLSATILYEILLGKATLYAVLVSTLVVMAMVKRKNSSR

SEQ ID NO: 16 - protein, 306 aa, synthetic construct
  REGION 1..306: note = ht27M1128 b chain
MLLLLLLLGPGSGLGAVVSQHPSWVICKSGTSVKIECRSLDFQATTMFWYRQFPKQSLMLMATSNEGSKATYEQGVEKDKFLINHASLTLSTLTVTSAHPEDSSFYICLAREPGQGPYEQYFGPGTRLTVTEDLRNVTPPKVSLFEPSKAEIANKQKATLVCLARGFFPDHVELSWWVNGKEVHSGVCTDPQAYKESNYSYCLSSRLRVSATFWHNPRNHFRCQVQFHGLSEEDKWPEGSPKPVTQNISAEAWGRADCGITSASYQQGVLSATILYEILLGKATLYAVLVSTLVVMAMVKRKNSSR

SEQ ID NO: 17 - protein, 306 aa, synthetic construct
  REGION 1..306: note = ht27M1166 b chain
MLLLLLLLGPGSGLGAVVSQHPSWVICKSGTSVKIECRSLDFQATTMFWYRQFPKQSLMLMATSNEGSKATYEQGVEKDKFLINHASLTLSTLTVTSAHPEDSSFYICQAREPGQGPYEQYFGPGTRLTVTEDLRNVTPPKVSLFEPSKAEIANKQKATLVCLARGFFPDHVELSWWVNGKEVHSGVCTDPQAYKESNYSYCLSSRLRVSATFWHNPRNHFRCQVQFHGLSEEDKWPEGSPKPVTQNISAEAWGRADCGITSASYQQGVLSATILYEILLGKATLYAVLVSTLVVMAMVKRKNSSR

SEQ ID NO: 18 - protein, 306 aa, synthetic construct
  REGION 1..306: note = ht27M1169 b chain
MLLLLLLLGPGSGLGAVVSQHPSWVICKSGTSVKIECRSLDFQATTMFWYRQFPKQSLMLMATSNEGSKATYEQGVEKDKFLINHASLTLSTLTVTSAHPEDSSFYICNAREPGQGPYEQYFGPGTRLTVTEDLRNVTPPKVSLFEPSKAEIANKQKATLVCLARGFFPDHVELSWWVNGKEVHSGVCTDPQAYKESNYSYCLSSRLRVSATFWHNPRNHFRCQVQFHGLSEEDKWPEGSPKPVTQNISAEAWGRADCGITSASYQQGVLSATILYEILLGKATLYAVLVSTLVVMAMVKRKNSSR

SEQ ID NO: 19 - protein, 306 aa, synthetic construct
  REGION 1..306: note = ht27M1170 b chain
MLLLLLLLGPGSGLGAVVSQHPSWVICKSGTSVKIECRSLDFQATTMFWYRQFPKQSLMLMATSNEGSKATYEQGVEKDKFLINHASLTLSTLTVTSAHPEDSSFYICHAREPGQGPYEQYFGPGTRLTVTEDLRNVTPPKVSLFEPSKAEIANKQKATLVCLARGFFPDHVELSWWVNGKEVHSGVCTDPQAYKESNYSYCLSSRLRVSATFWHNPRNHFRCQVQFHGLSEEDKWPEGSPKPVTQNISAEAWGRADCGITSASYQQGVLSATILYEILLGKATLYAVLVSTLVVMAMVKRKNSSR

SEQ ID NO: 20 - protein, 269 aa, synthetic construct
  REGION 1..269: note = ht27M1226 a chain
MKTFAGFSFLFLWLQLDCMSRGEDVEQSLFLSVREGDSSVINCTYTDSLSTYLYWYKQEPGAGLQLLTYIFSNMDMKQDQRLTVLLNKKDKHLSLRIADTQTGDSAIYFCAGSGGGTDKLIFGTGTRLQVFPNIQNPEPAVYQLKDPRSQDSTLCLFTDFDSQINVPKTMESGTFITDKCVLDMKAMDSKSNGAIAWSNQTSFTCQDIFKETNATYPSSDVPCDATLTEKSFETDMNLNFQNLLVIVLRILLLKVAGFNLLMTLRLWSS

SEQ ID NO: 21 - protein, 269 aa, synthetic construct
  REGION 1..269: note = ht27M1240 a chain
MKTFAGFSFLFLWLQLDCMSRGEDVEQSLFLSVREGDSSVINCTYTDSSMTYLYWYKQEPGAGLQLLTYIFSNMDMKQDQRLTVLLNKKDKHLSLRIADTQTGDSAIYFCAGSGGGTDKLIFGTGTRLQVFPNIQNPEPAVYQLKDPRSQDSTLCLFTDFDSQINVPKTMESGTFITDKCVLDMKAMDSKSNGAIAWSNQTSFTCQDIFKETNATYPSSDVPCDATLTEKSFETDMNLNFQNLLVIVLRILLLKVAGFNLLMTLRLWSS

SEQ ID NO: 22 - protein, 269 aa, synthetic construct
  REGION 1..269: note = ht27M1243 a chain
MKTFAGFSFLFLWLQLDCMSRGEDVEQSLFLSVREGDSSVINCTYTDSSLTYLYWYKQEPGAGLQLLTYIFSNMDMKQDQRLTVLLNKKDKHLSLRIADTQTGDSAIYFCAGSGGGTDKLIFGTGTRLQVFPNIQNPEPAVYQLKDPRSQDSTLCLFTDFDSQINVPKTMESGTFITDKCVLDMKAMDSKSNGAIAWSNQTSFTCQDIFKETNATYPSSDVPCDATLTEKSFETDMNLNFQNLLVIVLRILLLKVAGFNLLMTLRLWSS

SEQ ID NO: 23 - protein, 269 aa, synthetic construct
  REGION 1..269: note = ht27M1245 a chain
MKTFAGFSFLFLWLQLDCMSRGEDVEQSLFLSVREGDSSVINCTYTDSSQTYLYWYKQEPGAGLQLLTYIFSNMDMKQDQRLTVLLNKKDKHLSLRIADTQTGDSAIYFCAGSGGGTDKLIFGTGTRLQVFPNIQNPEPAVYQLKDPRSQDSTLCLFTDFDSQINVPKTMESGTFITDKCVLDMKAMDSKSNGAIAWSNQTSFTCQDIFKETNATYPSSDVPCDATLTEKSFETDMNLNFQNLLVIVLRILLLKVAGFNLLMTLRLWSS

SEQ ID NO: 24 - protein, 6 aa, synthetic construct
  REGION 1..6: note = WT ht27 CDR1b
DFQATT

SEQ ID NO: 25 - protein, 7 aa, synthetic construct
  REGION 1..7: note = WT ht27 CDR2b
SNEGSKA

SEQ ID NO: 26 - protein, 13 aa, synthetic construct
  REGION 1..13: note = WT ht27 CDR3b
SAREPGQGPYEQY

SEQ ID NO: 27 - protein, 6 aa, synthetic construct
  REGION 1..6: note = WT ht27 CDR1a
DSSSTY

SEQ ID NO: 28 - protein, 7 aa, synthetic construct
  REGION 1..7: note = WT ht27 CDR2a
IFSNMDM

SEQ ID NO: 29 - protein, 11 aa, synthetic construct
  REGION 1..11: note = WT ht27 CDR3a
AGSGGGTDKLI

SEQ ID NO: 30 - protein, 7 aa, synthetic construct
  REGION 1..7: note = ht27M1001 CDR2b
SDYQTCV

SEQ ID NO: 31 - protein, 13 aa, synthetic construct
  REGION 1..13: note = ht27M1002 CDR3b
SAREPGGGPYEQY

SEQ ID NO: 32 - protein, 13 aa, synthetic construct
  REGION 1..13: note = ht27M1003 CDR3b
SAREPGSGPYEQY

SEQ ID NO: 33 - protein, 13 aa, synthetic construct
  REGION 1..13: note = ht27M1004 CDR3b
SAREPGQGPFEQY

SEQ ID NO: 34 - protein, 13 aa, synthetic construct
  REGION 1..13: note = ht27M1005 CDR3b
SAREPGQGPLEQY

SEQ ID NO: 35 - protein, 13 aa, synthetic construct
  REGION 1..13: note = ht27M1006 CDR3b
SAREPGQGPWEQY

SEQ ID NO: 36 - protein, 13 aa, synthetic construct
  REGION 1..13: note = ht27M1012 CDR3b
SAREPGGGPFEQY

SEQ ID NO: 37 - protein, 13 aa, synthetic construct
  REGION 1..13: note = ht27M1013 CDR3b
SAREPGSGPFEQY

SEQ ID NO: 38 - protein, 13 aa, synthetic construct
  REGION 1..13: note = ht27M1128 CDR3b
LAREPGQGPYEQY

SEQ ID NO: 39 - protein, 13 aa, synthetic construct
  REGION 1..13: note = ht27M1166 CDR3b
QAREPGQGPYEQY

SEQ ID NO: 40 - protein, 13 aa, synthetic construct
  REGION 1..13: note = ht27M1169 CDR3b
NAREPGQGPYEQY

SEQ ID NO: 41 - protein, 13 aa, synthetic construct
  REGION 1..13: note = ht27M1170 CDR3b
HAREPGQGPYEQY

SEQ ID NO: 42 - protein, 6 aa, synthetic construct
  REGION 1..6: note = ht27M1226 CDR1a
DSLSTY

SEQ ID NO: 43 - protein, 6 aa, synthetic construct
  REGION 1..6: note = ht27M1240 CDR1a
DSSMTY

SEQ ID NO: 44 - protein, 6 aa, synthetic construct
  REGION 1..6: note = ht27M1243 CDR1a
DSSLTY

SEQ ID NO: 45 - protein, 6 aa, synthetic construct
  REGION 1..6: note = ht27M1245 CDR1a
DSSQTY

SEQ ID NO: 46 - protein, 113 aa, synthetic construct
  REGION 1..113: note = WT ht27 Va
RGEDVEQSLFLSVREGDSSVINCTYTDSSSTYLYWYKQEPGAGLQLLTYIFSNMDMKQDQRLTVLLNKKDKHLSLRIADTQTGDSAIYFCAGSGGGTDKLIFGTGTRLQVFPN

SEQ ID NO: 47 - protein, 118 aa, synthetic construct
  REGION 1..118: note = WT ht27 Vb
GAVVSQHPSWVICKSGTSVKIECRSLDFQATTMFWYRQFPKQSLMLMATSNEGSKATYEQGVEKDKFLINHASLTLSTLTVTSAHPEDSSFYICSAREPGQGPYEQYFGPGTRLTVTE

SEQ ID NO: 48 - protein, 118 aa, synthetic construct
  REGION 1..118: note = ht27M1001 Vb
GAVVSQHPSWVICKSGTSVKIECRSLDFQATTMFWYRQFPKQSLMLMATSDYQTCVTYEQGVEKDKFLINHASLTLSTLTVTSAHPEDSSFYICSAREPGQGPYEQYFGPGTRLTVTE

SEQ ID NO: 49 - protein, 118 aa, synthetic construct
  REGION 1..118: note = ht27M1002 Vb
GAVVSQHPSWVICKSGTSVKIECRSLDFQATTMFWYRQFPKQSLMLMATSNEGSKATYEQGVEKDKFLINHASLTLSTLTVTSAHPEDSSFYICSAREPGGGPYEQYFGPGTRLTVTE

SEQ ID NO: 50 - protein, 118 aa, synthetic construct
  REGION 1..118: note = ht27M1003 Vb
GAVVSQHPSWVICKSGTSVKIECRSLDFQATTMFWYRQFPKQSLMLMATSNEGSKATYEQGVEKDKFLINHASLTLSTLTVTSAHPEDSSFYICSAREPGSGPYEQYFGPGTRLTVTE

SEQ ID NO: 51 - protein, 118 aa, synthetic construct
  REGION 1..118: note = ht27M1004 Vb
GAVVSQHPSWVICKSGTSVKIECRSLDFQATTMFWYRQFPKQSLMLMATSNEGSKATYEQGVEKDKFLINHASLTLSTLTVTSAHPEDSSFYICSAREPGQGPFEQYFGPGTRLTVTE

SEQ ID NO: 52 - protein, 118 aa, synthetic construct
  REGION 1..118: note = ht27M1005 Vb
GAVVSQHPSWVICKSGTSVKIECRSLDFQATTMFWYRQFPKQSLMLMATSNEGSKATYEQGVEKDKFLINHASLTLSTLTVTSAHPEDSSFYICSAREPGQGPLEQYFGPGTRLTVTE

SEQ ID NO: 53 - protein, 118 aa, synthetic construct
  REGION 1..118: note = ht27M1006 Vb
GAVVSQHPSWVICKSGTSVKIECRSLDFQATTMFWYRQFPKQSLMLMATSNEGSKATYEQGVEKDKFLINHASLTLSTLTVTSAHPEDSSFYICSAREPGQGPWEQYFGPGTRLTVTE

SEQ ID NO: 54 - protein, 118 aa, synthetic construct
  REGION 1..118: note = ht27M1009 Vb
GAVVSQHPSWVICKSGTSVKIECRSLDFQATTMFWYRQFPKQSLMLMATSDYQTCVTYEQGVEKDKFLINHASLTLSTLTVTSAHPEDSSFYICSAREPGQGPFEQYFGPGTRLTVTE

SEQ ID NO: 55 - protein, 118 aa, synthetic construct
  REGION 1..118: note = ht27M1010 Vb
GAVVSQHPSWVICKSGTSVKIECRSLDFQATTMFWYRQFPKQSLMLMATSDYQTCVTYEQGVEKDKFLINHASLTLSTLTVTSAHPEDSSFYICSAREPGQGPLEQYFGPGTRLTVTE

SEQ ID NO: 56 - protein, 118 aa, synthetic construct
  REGION 1..118: note = ht27M1011 Vb
GAVVSQHPSWVICKSGTSVKIECRSLDFQATTMFWYRQFPKQSLMLMATSDYQTCVTYEQGVEKDKFLINHASLTLSTLTVTSAHPEDSSFYICSAREPGQGPWEQYFGPGTRLTVTE

SEQ ID NO: 57 - protein, 118 aa, synthetic construct
  REGION 1..118: note = ht27M1012 Vb
GAVVSQHPSWVICKSGTSVKIECRSLDFQATTMFWYRQFPKQSLMLMATSNEGSKATYEQGVEKDKFLINHASLTLSTLTVTSAHPEDSSFYICSAREPGGGPFEQYFGPGTRLTVTE

SEQ ID NO: 58 - protein, 118 aa, synthetic construct
  REGION 1..118: note = ht27M1013 Vb
GAVVSQHPSWVICKSGTSVKIECRSLDFQATTMFWYRQFPKQSLMLMATSNEGSKATYEQGVEKDKFLINHASLTLSTLTVTSAHPEDSSFYICSAREPGSGPFEQYFGPGTRLTVTE

SEQ ID NO: 59 - protein, 118 aa, synthetic construct
  REGION 1..118: note = ht27M1018 Vb
GAVVSQHPSWVICKSGTSVKIECRSLDFQATTMFWYRQFPKQSLMLMATSDYQTCVTYEQGVEKDKFLINHASLTLSTLTVTSAHPEDSSFYICSAREPGGGPFEQYFGPGTRLTVTE

SEQ ID NO: 60 - protein, 118 aa, synthetic construct
  REGION 1..118: note = ht27M1019 Vb
GAVVSQHPSWVICKSGTSVKIECRSLDFQATTMFWYRQFPKQSLMLMATSDYQTCVTYEQGVEKDKFLINHASLTLSTLTVTSAHPEDSSFYICSAREPGSGPFEQYFGPGTRLTVTE

SEQ ID NO: 61 - protein, 118 aa, synthetic construct
  REGION 1..118: note = ht27M1128 Vb
GAVVSQHPSWVICKSGTSVKIECRSLDFQATTMFWYRQFPKQSLMLMATSNEGSKATYEQGVEKDKFLINHASLTLSTLTVTSAHPEDSSFYICLAREPGQGPYEQYFGPGTRLTVTE

SEQ ID NO: 62 - protein, 118 aa, synthetic construct
  REGION 1..118: note = ht27M1166 Vb
GAVVSQHPSWVICKSGTSVKIECRSLDFQATTMFWYRQFPKQSLMLMATSNEGSKATYEQGVEKDKFLINHASLTLSTLTVTSAHPEDSSFYICQAREPGQGPYEQYFGPGTRLTVTE

SEQ ID NO: 63 - protein, 118 aa, synthetic construct
  REGION 1..118: note = ht27M1169 Vb
GAVVSQHPSWVICKSGTSVKIECRSLDFQATTMFWYRQFPKQSLMLMATSNEGSKATYEQGVEKDKFLINHASLTLSTLTVTSAHPEDSSFYICNAREPGQGPYEQYFGPGTRLTVTE

SEQ ID NO: 64 - protein, 118 aa, synthetic construct
  REGION 1..118: note = ht27M1170 Vb
GAVVSQHPSWVICKSGTSVKIECRSLDFQATTMFWYRQFPKQSLMLMATSNEGSKATYEQGVEKDKFLINHASLTLSTLTVTSAHPEDSSFYICHAREPGQGPYEQYFGPGTRLTVTE

SEQ ID NO: 65 - protein, 113 aa, synthetic construct
  REGION 1..113: note = ht27M1226 Va
RGEDVEQSLFLSVREGDSSVINCTYTDSLSTYLYWYKQEPGAGLQLLTYIFSNMDMKQDQRLTVLLNKKDKHLSLRIADTQTGDSAIYFCAGSGGGTDKLIFGTGTRLQVFPN

SEQ ID NO: 66 - protein, 113 aa, synthetic construct
  REGION 1..113: note = ht27M1240 Va
RGEDVEQSLFLSVREGDSSVINCTYTDSSMTYLYWYKQEPGAGLQLLTYIFSNMDMKQDQRLTVLLNKKDKHLSLRIADTQTGDSAIYFCAGSGGGTDKLIFGTGTRLQVFPN

SEQ ID NO: 67 - protein, 113 aa, synthetic construct
  REGION 1..113: note = ht27M1243 Va
RGEDVEQSLFLSVREGDSSVINCTYTDSSLTYLYWYKQEPGAGLQLLTYIFSNMDMKQDQRLTVLLNKKDKHLSLRIADTQTGDSAIYFCAGSGGGTDKLIFGTGTRLQVFPN

SEQ ID NO: 68 - protein, 113 aa, synthetic construct
  REGION 1..113: note = ht27M1245 Va
RGEDVEQSLFLSVREGDSSVINCTYTDSSQTYLYWYKQEPGAGLQLLTYIFSNMDMKQDQRLTVLLNKKDKHLSLRIADTQTGDSAIYFCAGSGGGTDKLIFGTGTRLQVFPN

SEQ ID NO: 69 - protein, 269 aa, synthetic construct
  REGION 1..269: note = WT ht27 a chain
MKTFAGFSFLFLWLQLDCMSRGEDVEQSLFLSVREGDSSVINCTYTDSSSTYLYWYKQEPGAGLQLLTYIFSNMDMKQDQRLTVLLNKKDKHLSLRIADTQTGDSAIYFCAGSGGGTDKLIFGTGTRLQVFPNIQNPEPAVYQLKDPRSQDSTLCLFTDFDSQINVPKTMESGTFITDKCVLDMKAMDSKSNGAIAWSNQTSFTCQDIFKETNATYPSSDVPCDATLTEKSFETDMNLNFQNLLVIVLRILLLKVAGFNLLMTLRLWSS

SEQ ID NO: 70 - protein, 306 aa, synthetic construct
  REGION 1..306: note = WT ht27 b chain
MLLLLLLLGPGSGLGAVVSQHPSWVICKSGTSVKIECRSLDFQATTMFWYRQFPKQSLMLMATSNEGSKATYEQGVEKDKFLINHASLTLSTLTVTSAHPEDSSFYICSAREPGQGPYEQYFGPGTRLTVTEDLRNVTPPKVSLFEPSKAEIANKQKATLVCLARGFFPDHVELSWWVNGKEVHSGVCTDPQAYKESNYSYCLSSRLRVSATFWHNPRNHFRCQVQFHGLSEEDKWPEGSPKPVTQNISAEAWGRADCGITSASYQQGVLSATILYEILLGKATLYAVLVSTLVVMAMVKRKNSSR

SEQ ID NO: 71 - protein, 136 aa, synthetic construct
  REGION 1..136: note = TCR a chain constant region
IQNPEPAVYQLKDPRSQDSTLCLFTDFDSQINVPKTMESGTFITDKCVLDMKAMDSKSNGAIAWSNQTSFTCQDIFKETNATYPSSDVPCDATLTEKSFETDMNLNFQNLLVIVLRILLLKVAGFNLLMTLRLWSS

SEQ ID NO: 72 - protein, 174 aa, synthetic construct
  REGION 1..174: note = TCR b chain constant region
DLRNVTPPKVSLFEPSKAEIANKQKATLVCLARGFFPDHVELSWWVNGKEVHSGVCTDPQAYKESNYSYCLSSRLRVSATFWHNPRNHFRCQVQFHGLSEEDKWPEGSPKPVTQNISAEAWGRADCGITSASYQQGVLSATILYEILLGKATLYAVLVSTLVVMAMVKRKNSSR

SEQ ID NO: 73 - protein, 19 aa, synthetic construct
  REGION 1..19: note = 2A self-cleaving peptide
ATNFSLLKQAGDVEENPGP

SEQ ID NO: 74 - protein, 20 aa, synthetic construct
  REGION 1..20: note = a chain signal peptide sequence
MKTFAGFSFLFLWLQLDCMS

SEQ ID NO: 75 - protein, 14 aa, synthetic construct
  REGION 1..14: note = b chain signal peptide sequence
MLLLLLLLGPGSGL

SEQ ID NO: 76 - protein, 7 aa, synthetic construct
  REGION 1..7: note = ht27M1285 CDR2a
IFSFMDM

SEQ ID NO: 77 - protein, 113 aa, synthetic construct
  REGION 1..113: note = ht27M1285 Va
RGEDVEQSLFLSVREGDSSVINCTYTDSSSTYLYWYKQEPGAGLQLLTYIFSFMDMKQDQRLTVLLNKKDKHLSLRIADTQTGDSAIYFCAGSGGGTDKLIFGTGTRLQVFPN

SEQ ID NO: 78 - protein, 269 aa, synthetic construct
  REGION 1..269: note = ht27M1285 a chain
MKTFAGFSFLFLWLQLDCMSRGEDVEQSLFLSVREGDSSVINCTYTDSSSTYLYWYKQEPGAGLQLLTYIFSFMDMKQDQRLTVLLNKKDKHLSLRIADTQTGDSAIYFCAGSGGGTDKLIFGTGTRLQVFPNIQNPEPAVYQLKDPRSQDSTLCLFTDFDSQINVPKTMESGTFITDKCVLDMKAMDSKSNGAIAWSNQTSFTCQDIFKETNATYPSSDVPCDATLTEKSFETDMNLNFQNLLVIVLRILLLKVAGFNLLMTLRLWSS

SEQ ID NO: 79 - protein, 12 aa, synthetic construct
  REGION 1..12: note = ht27M1290 CDR3b
SARVNDGTYEQY

SEQ ID NO: 80 - protein, 117 aa, synthetic construct
  REGION 1..117: note = ht27M1290 Vb
GAVVSQHPSWVICKSGTSVKIECRSLDFQATTMFWYRQFPKQSLMLMATSNEGSKATYEQGVEKDKFLINHASLTLSTLTVTSAHPEDSSFYICSARVNDGTYEQYFGPGTRLTVTE

SEQ ID NO: 81 - protein, 305 aa, synthetic construct
  REGION 1..305: note = ht27M1290 b chain
MLLLLLLLGPGSGLGAVVSQHPSWVICKSGTSVKIECRSLDFQATTMFWYRQFPKQSLMLMATSNEGSKATYEQGVEKDKFLINHASLTLSTLTVTSAHPEDSSFYICSARVNDGTYEQYFGPGTRLTVTEDLRNVTPPKVSLFEPSKAEIANKQKATLVCLARGFFPDHVELSWWVNGKEVHSGVCTDPQAYKESNYSYCLSSRLRVSATFWHNPRNHFRCQVQFHGLSEEDKWPEGSPKPVTQNISAEAWGRADCGITSASYQQGVLSATILYEILLGKATLYAVLVSTLVVMAMVKRKNSSR

SEQ ID NO: 82 - protein, 6 aa, synthetic construct
  REGION 1..6: note = ht27M1387 CDR1b
DFPIER

SEQ ID NO: 83 - protein, 118 aa, synthetic construct
  REGION 1..118: note = ht27M1387 Vb
GAVVSQHPSWVICKSGTSVKIECRSLDFPIERMFWYRQFPKQSLMLMATSNEGSKATYEQGVEKDKFLINHASLTLSTLTVTSAHPEDSSFYICSAREPGQGPYEQYFGPGTRLTVTE

SEQ ID NO: 84 - protein, 306 aa, synthetic construct
  REGION 1..306: note = ht27M1387 b chain
MLLLLLLLGPGSGLGAVVSQHPSWVICKSGTSVKIECRSLDFPIERMFWYRQFPKQSLMLMATSNEGSKATYEQGVEKDKFLINHASLTLSTLTVTSAHPEDSSFYICSAREPGQGPYEQYFGPGTRLTVTEDLRNVTPPKVSLFEPSKAEIANKQKATLVCLARGFFPDHVELSWWVNGKEVHSGVCTDPQAYKESNYSYCLSSRLRVSATFWHNPRNHFRCQVQFHGLSEEDKWPEGSPKPVTQNISAEAWGRADCGITSASYQQGVLSATILYEILLGKATLYAVLVSTLVVMAMVKRKNSSR

SEQ ID NO: 85 - protein, 7 aa, synthetic construct
  REGION 1..7: note = ht27M1398 CDR2b
TNLPSKA

SEQ ID NO: 86 - protein, 118 aa, synthetic construct
  REGION 1..118: note = ht27M1398 Vb
GAVVSQHPSWVICKSGTSVKIECRSLDFQATTMFWYRQFPKQSLMLMATTNLPSKATYEQGVEKDKFLINHASLTLSTLTVTSAHPEDSSFYICSAREPGQGPYEQYFGPGTRLTVTE

SEQ ID NO: 87 - protein, 306 aa, synthetic construct
  REGION 1..306: note = ht27M1398 b chain
MLLLLLLLGPGSGLGAVVSQHPSWVICKSGTSVKIECRSLDFQATTMFWYRQFPKQSLMLMATTNLPSKATYEQGVEKDKFLINHASLTLSTLTVTSAHPEDSSFYICSAREPGQGPYEQYFGPGTRLTVTEDLRNVTPPKVSLFEPSKAEIANKQKATLVCLARGFFPDHVELSWWVNGKEVHSGVCTDPQAYKESNYSYCLSSRLRVSATFWHNPRNHFRCQVQFHGLSEEDKWPEGSPKPVTQNISAEAWGRADCGITSASYQQGVLSATILYEILLGKATLYAVLVSTLVVMAMVKRKNSSR

SEQ ID NO: 88 - protein, 7 aa, synthetic construct
  REGION 1..7: note = ht27M1401 CDR2b
TQPLSKA

SEQ ID NO: 89 - protein, 118 aa, synthetic construct
  REGION 1..118: note = ht27M1401 Vb
GAVVSQHPSWVICKSGTSVKIECRSLDFQATTMFWYRQFPKQSLMLMATTQPLSKATYEQGVEKDKFLINHASLTLSTLTVTSAHPEDSSFYICSAREPGQGPYEQYFGPGTRLTVTE

SEQ ID NO: 90 - protein, 306 aa, synthetic construct
  REGION 1..306: note = ht27M1401 b chain
MLLLLLLLGPGSGLGAVVSQHPSWVICKSGTSVKIECRSLDFQATTMFWYRQFPKQSLMLMATTQPLSKATYEQGVEKDKFLINHASLTLSTLTVTSAHPEDSSFYICSAREPGQGPYEQYFGPGTRLTVTEDLRNVTPPKVSLFEPSKAEIANKQKATLVCLARGFFPDHVELSWWVNGKEVHSGVCTDPQAYKESNYSYCLSSRLRVSATFWHNPRNHFRCQVQFHGLSEEDKWPEGSPKPVTQNISAEAWGRADCGITSASYQQGVLSATILYEILLGKATLYAVLVSTLVVMAMVKRKNSSR

SEQ ID NO: 91 - protein, 7 aa, synthetic construct
  REGION 1..7: note = ht27M1457 CDR2b
TDYGSKA

SEQ ID NO: 92 - protein, 118 aa, synthetic construct
  REGION 1..118: note = ht27M1457 Vb
GAVVSQHPSWVICKSGTSVKIECRSLDFQATTMFWYRQFPKQSLMLMATTDYGSKATYEQGVEKDKFLINHASLTLSTLTVTSAHPEDSSFYICSAREPGQGPYEQYFGPGTRLTVTE

SEQ ID NO: 93 - protein, 306 aa, synthetic construct
  REGION 1..306: note = ht27M1457 b chain
MLLLLLLLGPGSGLGAVVSQHPSWVICKSGTSVKIECRSLDFQATTMFWYRQFPKQSLMLMATTDYGSKATYEQGVEKDKFLINHASLTLSTLTVTSAHPEDSSFYICSAREPGQGPYEQYFGPGTRLTVTEDLRNVTPPKVSLFEPSKAEIANKQKATLVCLARGFFPDHVELSWWVNGKEVHSGVCTDPQAYKESNYSYCLSSRLRVSATFWHNPRNHFRCQVQFHGLSEEDKWPEGSPKPVTQNISAEAWGRADCGITSASYQQGVLSATILYEILLGKATLYAVLVSTLVVMAMVKRKNSSR

SEQ ID NO: 94 - protein, 13 aa, synthetic construct
  REGION 1..13: note = ht27M1557 CDR3b
SAREPGQEHLIQY

SEQ ID NO: 95 - protein, 118 aa, synthetic construct
  REGION 1..118: note = ht27M1557 Vb
GAVVSQHPSWVICKSGTSVKIECRSLDFQATTMFWYRQFPKQSLMLMATSNEGSKATYEQGVEKDKFLINHASLTLSTLTVTSAHPEDSSFYICSAREPGQEHLIQYFGPGTRLTVTE

SEQ ID NO: 96 - protein, 306 aa, synthetic construct
  REGION 1..306: note = ht27M1557 b chain
MLLLLLLLGPGSGLGAVVSQHPSWVICKSGTSVKIECRSLDFQATTMFWYRQFPKQSLMLMATSNEGSKATYEQGVEKDKFLINHASLTLSTLTVTSAHPEDSSFYICSAREPGQEHLIQYFGPGTRLTVTEDLRNVTPPKVSLFEPSKAEIANKQKATLVCLARGFFPDHVELSWWVNGKEVHSGVCTDPQAYKESNYSYCLSSRLRVSATFWHNPRNHFRCQVQFHGLSEEDKWPEGSPKPVTQNISAEAWGRADCGITSASYQQGVLSATILYEILLGKATLYAVLVSTLVVMAMVKRKNSSR

SEQ ID NO: 97 - protein, 6 aa, synthetic construct
  REGION 1..6: note = ht27M1374 CDR1a
DSTDIL

SEQ ID NO: 98 - protein, 113 aa, synthetic construct
  REGION 1..113: note = ht27M1374 Va
RGEDVEQSLFLSVREGDSSVINCTYTDSTDILLYWYKQEPGAGLQLLTYIFSNMDMKQDQRLTVLLNKKDKHLSLRIADTQTGDSAIYFCAGSGGGTDKLIFGTGTRLQVFPN

SEQ ID NO: 99 - protein, 269 aa, synthetic construct
  REGION 1..269: note = ht27M1374 a chain
MKTFAGFSFLFLWLQLDCMSRGEDVEQSLFLSVREGDSSVINCTYTDSTDILLYWYKQEPGAGLQLLTYIFSNMDMKQDQRLTVLLNKKDKHLSLRIADTQTGDSAIYFCAGSGGGTDKLIFGTGTRLQVFPNIQNPEPAVYQLKDPRSQDSTLCLFTDFDSQINVPKTMESGTFITDKCVLDMKAMDSKSNGAIAWSNQTSFTCQDIFKETNATYPSSDVPCDATLTEKSFETDMNLNFQNLLVIVLRILLLKVAGFNLLMTLRLWSS

SEQ ID NO: 100 - protein, 6 aa, synthetic construct
  REGION 1..6: note = ht27M1378 CDR1a
DYLSTY

SEQ ID NO: 101 - protein, 113 aa, synthetic construct
  REGION 1..113: note = ht27M1378 Va
RGEDVEQSLFLSVREGDSSVINCTYADYLSTYLYWYKQEPGAGLQLLTYIFSNMDMKQDQRLTVLLNKKDKHLSLRIADTQTGDSAIYFCAGSGGGTDKLIFGTGTRLQVFPN

SEQ ID NO: 102 - protein, 269 aa, synthetic construct
  REGION 1..269: note = ht27M1378 a chain
MKTFAGFSFLFLWLQLDCMSRGEDVEQSLFLSVREGDSSVINCTYADYLSTYLYWYKQEPGAGLQLLTYIFSNMDMKQDQRLTVLLNKKDKHLSLRIADTQTGDSAIYFCAGSGGGTDKLIFGTGTRLQVFPNIQNPEPAVYQLKDPRSQDSTLCLFTDFDSQINVPKTMESGTFITDKCVLDMKAMDSKSNGAIAWSNQTSFTCQDIFKETNATYPSSDVPCDATLTEKSFETDMNLNFQNLLVIVLRILLLKVAGFNLLMTLRLWSS

SEQ ID NO: 103 - protein, 6 aa, synthetic construct
  REGION 1..6: note = ht27M1381, A1A2-M01-612 CDR1a
DPYSTY

SEQ ID NO: 104 - protein, 113 aa, synthetic construct
  REGION 1..113: note = ht27M1381 Va
RGEDVEQSLFLSVREGDSSVINCTYVDPYSTYLYWYKQEPGAGLQLLTYIFSNMDMKQDQRLTVLLNKKDKHLSLRIADTQTGDSAIYFCAGSGGGTDKLIFGTGTRLQVFPN

SEQ ID NO: 105 - protein, 269 aa, synthetic construct
  REGION 1..269: note = ht27M1381 a chain
MKTFAGFSFLFLWLQLDCMSRGEDVEQSLFLSVREGDSSVINCTYVDPYSTYLYWYKQEPGAGLQLLTYIFSNMDMKQDQRLTVLLNKKDKHLSLRIADTQTGDSAIYFCAGSGGGTDKLIFGTGTRLQVFPNIQNPEPAVYQLKDPRSQDSTLCLFTDFDSQINVPKTMESGTFITDKCVLDMKAMDSKSNGAIAWSNQTSFTCQDIFKETNATYPSSDVPCDATLTEKSFETDMNLNFQNLLVIVLRILLLKVAGFNLLMTLRLWSS

SEQ ID NO: 106 - protein, 7 aa, synthetic construct
  REGION 1..7: note = ht27M1360 CDR2a
IFGFDTM

SEQ ID NO: 107 - protein, 113 aa, synthetic construct
  REGION 1..113: note = ht27M1360 Va
RGEDVEQSLFLSVREGDSSVINCTYTDSSSTYLYWYKQEPGAGLQLLTYIFGFDTMKQDQRLTVLLNKKDKHLSLRIADTQTGDSAIYFCAGSGGGTDKLIFGTGTRLQVFPN

SEQ ID NO: 108 - protein, 269 aa, synthetic construct
  REGION 1..269: note = ht27M1360 a chain
MKTFAGFSFLFLWLQLDCMSRGEDVEQSLFLSVREGDSSVINCTYTDSSSTYLYWYKQEPGAGLQLLTYIFGFDTMKQDQRLTVLLNKKDKHLSLRIADTQTGDSAIYFCAGSGGGTDKLIFGTGTRLQVFPNIQNPEPAVYQLKDPRSQDSTLCLFTDFDSQINVPKTMESGTFITDKCVLDMKAMDSKSNGAIAWSNQTSFTCQDIFKETNATYPSSDVPCDATLTEKSFETDMNLNFQNLLVIVLRILLLKVAGFNLLMTLRLWSS

SEQ ID NO: 109 - protein, 7 aa, synthetic construct
  REGION 1..7: note = ht27M1362 CDR2a
IFIFQYM

SEQ ID NO: 110 - protein, 113 aa, synthetic construct
  REGION 1..113: note = ht27M1362 Va
RGEDVEQSLFLSVREGDSSVINCTYTDSSSTYLYWYKQEPGAGLQLLTYIFIFQYMKQDQRLTVLLNKKDKHLSLRIADTQTGDSAIYFCAGSGGGTDKLIFGTGTRLQVFPN

SEQ ID NO: 111 - protein, 269 aa, synthetic construct
  REGION 1..269: note = ht27M1362 a chain
MKTFAGFSFLFLWLQLDCMSRGEDVEQSLFLSVREGDSSVINCTYTDSSSTYLYWYKQEPGAGLQLLTYIFIFQYMKQDQRLTVLLNKKDKHLSLRIADTQTGDSAIYFCAGSGGGTDKLIFGTGTRLQVFPNIQNPEPAVYQLKDPRSQDSTLCLFTDFDSQINVPKTMESGTFITDKCVLDMKAMDSKSNGAIAWSNQTSFTCQDIFKETNATYPSSDVPCDATLTEKSFETDMNLNFQNLLVIVLRILLLKVAGFNLLMTLRLWSS

SEQ ID NO: 112 - protein, 7 aa, synthetic construct
  REGION 1..7: note = ht27M1363 CDR2a
IFNTQDM

SEQ ID NO: 113 - protein, 113 aa, synthetic construct
  REGION 1..113: note = ht27M1363 Va
RGEDVEQSLFLSVREGDSSVINCTYTDSSSTYLYWYKQEPGAGLQLLTYIFNTQDMKQDQRLTVLLNKKDKHLSLRIADTQTGDSAIYFCAGSGGGTDKLIFGTGTRLQVFPN

SEQ ID NO: 114 - protein, 269 aa, synthetic construct
  REGION 1..269: note = ht27M1363 a chain
MKTFAGFSFLFLWLQLDCMSRGEDVEQSLFLSVREGDSSVINCTYTDSSSTYLYWYKQEPGAGLQLLTYIFNTQDMKQDQRLTVLLNKKDKHLSLRIADTQTGDSAIYFCAGSGGGTDKLIFGTGTRLQVFPNIQNPEPAVYQLKDPRSQDSTLCLFTDFDSQINVPKTMESGTFITDKCVLDMKAMDSKSNGAIAWSNQTSFTCQDIFKETNATYPSSDVPCDATLTEKSFETDMNLNFQNLLVIVLRILLLKVAGFNLLMTLRLWSS

SEQ ID NO: 115 - protein, 7 aa, synthetic construct
  REGION 1..7: note = ht27M1365 CDR2a
IFSFTYM

SEQ ID NO: 116 - protein, 113 aa, synthetic construct
  REGION 1..113: note = ht27M1365 Va
RGEDVEQSLFLSVREGDSSVINCTYTDSSSTYLYWYKQEPGAGLQLLTYIFSFTYMKQDQRLTVLLNKKDKHLSLRIADTQTGDSAIYFCAGSGGGTDKLIFGTGTRLQVFPN

SEQ ID NO: 117 - protein, 269 aa, synthetic construct
  REGION 1..269: note = ht27M1365 a chain
MKTFAGFSFLFLWLQLDCMSRGEDVEQSLFLSVREGDSSVINCTYTDSSSTYLYWYKQEPGAGLQLLTYIFSFTYMKQDQRLTVLLNKKDKHLSLRIADTQTGDSAIYFCAGSGGGTDKLIFGTGTRLQVFPNIQNPEPAVYQLKDPRSQDSTLCLFTDFDSQINVPKTMESGTFITDKCVLDMKAMDSKSNGAIAWSNQTSFTCQDIFKETNATYPSSDVPCDATLTEKSFETDMNLNFQNLLVIVLRILLLKVAGFNLLMTLRLWSS

SEQ ID NO: 118 - protein, 7 aa, synthetic construct
  REGION 1..7: note = ht27M1369 CDR2a
IFAFESM

SEQ ID NO: 119 - protein, 113 aa, synthetic construct
  REGION 1..113: note = ht27M1369 Va
RGEDVEQSLFLSVREGDSSVINCTYTDSSSTYLYWYKQEPGAGLQLLTYIFAFESMKQDQRLTVLLNKKDKHLSLRIADTQTGDSAIYFCAGSGGGTDKLIFGTGTRLQVFPN

SEQ ID NO: 120 - protein, 269 aa, synthetic construct
  REGION 1..269: note = ht27M1369 a chain
MKTFAGFSFLFLWLQLDCMSRGEDVEQSLFLSVREGDSSVINCTYTDSSSTYLYWYKQEPGAGLQLLTYIFAFESMKQDQRLTVLLNKKDKHLSLRIADTQTGDSAIYFCAGSGGGTDKLIFGTGTRLQVFPNIQNPEPAVYQLKDPRSQDSTLCLFTDFDSQINVPKTMESGTFITDKCVLDMKAMDSKSNGAIAWSNQTSFTCQDIFKETNATYPSSDVPCDATLTEKSFETDMNLNFQNLLVIVLRILLLKVAGFNLLMTLRLWSS

SEQ ID NO: 121 - protein, 7 aa, synthetic construct
  REGION 1..7: note = ht27M1414 CDR2a
TWPHMDM

SEQ ID NO: 122 - protein, 113 aa, synthetic construct
  REGION 1..113: note = ht27M1414 Va
RGEDVEQSLFLSVREGDSSVINCTYTDSSSTYLYWYKQEPGAGLQLLTYTWPHMDMKQDQRLTVLLNKKDKHLSLRIADTQTGDSAIYFCAGSGGGTDKLIFGTGTRLQVFPN

SEQ ID NO: 123 - protein, 269 aa, synthetic construct
  REGION 1..269: note = ht27M1414 a chain
MKTFAGFSFLFLWLQLDCMSRGEDVEQSLFLSVREGDSSVINCTYTDSSSTYLYWYKQEPGAGLQLLTYTWPHMDMKQDQRLTVLLNKKDKHLSLRIADTQTGDSAIYFCAGSGGGTDKLIFGTGTRLQVFPNIQNPEPAVYQLKDPRSQDSTLCLFTDFDSQINVPKTMESGTFITDKCVLDMKAMDSKSNGAIAWSNQTSFTCQDIFKETNATYPSSDVPCDATLTEKSFETDMNLNFQNLLVIVLRILLLKVAGFNLLMTLRLWSS

SEQ ID NO: 124 - protein, 7 aa, synthetic construct
  REGION 1..7: note = ht27M1418 CDR2a
GTWLMDM

SEQ ID NO: 125 - protein, 113 aa, synthetic construct
  REGION 1..113: note = ht27M1418 Va
RGEDVEQSLFLSVREGDSSVINCTYTDSSSTYLYWYKQEPGAGLQLLTYGTWLMDMKQDQRLTVLLNKKDKHLSLRIADTQTGDSAIYFCAGSGGGTDKLIFGTGTRLQVFPN

SEQ ID NO: 126 - protein, 269 aa, synthetic construct
  REGION 1..269: note = ht27M1418 a chain
MKTFAGFSFLFLWLQLDCMSRGEDVEQSLFLSVREGDSSVINCTYTDSSSTYLYWYKQEPGAGLQLLTYGTWLMDMKQDQRLTVLLNKKDKHLSLRIADTQTGDSAIYFCAGSGGGTDKLIFGTGTRLQVFPNIQNPEPAVYQLKDPRSQDSTLCLFTDFDSQINVPKTMESGTFITDKCVLDMKAMDSKSNGAIAWSNQTSFTCQDIFKETNATYPSSDVPCDATLTEKSFETDMNLNFQNLLVIVLRILLLKVAGFNLLMTLRLWSS

SEQ ID NO: 127 - protein, 7 aa, synthetic construct
  REGION 1..7: note = ht27M1436 CDR2a
TFWFMDM

SEQ ID NO: 128 - protein, 113 aa, synthetic construct
  REGION 1..113: note = ht27M1436 Va
RGEDVEQSLFLSVREGDSSVINCTYTDSSSTYLYWYKQEPGAGLQLLTYTFWFMDMKQDQRLTVLLNKKDKHLSLRIADTQTGDSAIYFCAGSGGGTDKLIFGTGTRLQVFPN

SEQ ID NO: 129 - protein, 269 aa, synthetic construct
  REGION 1..269: note = ht27M1436 a chain
MKTFAGFSFLFLWLQLDCMSRGEDVEQSLFLSVREGDSSVINCTYTDSSSTYLYWYKQEPGAGLQLLTYTFWFMDMKQDQRLTVLLNKKDKHLSLRIADTQTGDSAIYFCAGSGGGTDKLIFGTGTRLQVFPNIQNPEPAVYQLKDPRSQDSTLCLFTDFDSQINVPKTMESGTFITDKCVLDMKAMDSKSNGAIAWSNQTSFTCQDIFKETNATYPSSDVPCDATLTEKSFETDMNLNFQNLLVIVLRILLLKVAGFNLLMTLRLWSS

SEQ ID NO: 130 - protein, 6 aa, synthetic construct
  REGION 1..6: note = A1A2-M01-612 CDR1b
DFEATT

SEQ ID NO: 131 - protein, 13 aa, synthetic construct
  REGION 1..13: note = A1A2-M01-612 CDR3b
SAREPWDPWYEQY

SEQ ID NO: 132 - protein, 113 aa, synthetic construct
  REGION 1..113: note = A1A2-M01-612 Va
RGEDVEQSLFLSVREGDSSVINCTYVDPYSTYLYWYKQEPGAGLQLLTYIFSFMDMKQDQRLTVLLNKKDKHLSLRIADTQTGDSAIYFCAGSGGGTDKLIFGTGTRLQVFPN

SEQ ID NO: 133 - protein, 118 aa, synthetic construct
  REGION 1..118: note = A1A2-M01-612 Vb
GAVVSQHPSWVICKSGTSVKIECRSLDFEATTMFWYRQFPKQSLMLMATSNEGSKATYEQGVEKDKFLINHASLTLSTLTVTSAHPEDSSFYICSAREPWDPWYEQYFGPGTRLTVTE

SEQ ID NO: 134 - protein, 269 aa, synthetic construct
  REGION 1..269: note = A1A2-M01-612 a chain
MKTFAGFSFLFLWLQLDCMSRGEDVEQSLFLSVREGDSSVINCTYVDPYSTYLYWYKQEPGAGLQLLTYIFSFMDMKQDQRLTVLLNKKDKHLSLRIADTQTGDSAIYFCAGSGGGTDKLIFGTGTRLQVFPNIQNPEPAVYQLKDPRSQDSTLCLFTDFDSQINVPKTMESGTFITDKCVLDMKAMDSKSNGAIAWSNQTSFTCQDIFKETNATYPSSDVPCDATLTEKSFETDMNLNFQNLLVIVLRILLLKVAGFNLLMTLRLWSS

SEQ ID NO: 135 - protein, 304 aa, synthetic construct
  REGION 1..304: note = A1A2-M01-612 b chain
MLLLLLLLGPGSGLGAVVSQHPSWVICKSGTSVKIECRSLDFEATTMFWYRQFPKQSLMLMATSNEGSKATYEQGVEKDKFLINHASLTLSTLTVTSAHPEDSSFYICSAREPWDPWYEQYFGPGTRLTVTEDLRNVTPPKVSLFEPSKAEIANKQKATLVCLARGFFPDHVELSWWVNGKEVHSGVCTDPQAYKESNYSYCLSSRLRVSATFWHNPRNHFRCQVQFHGLSEEDKWPEGSPKPVTQNISAEAWGRADCGITSASYQQGVLSATILYEILLGKATLYAVLVSTLVVMAMVKRKNS

SEQ ID NO: 136 - protein, 113 aa, synthetic construct
  REGION 1..113: note = A1A2-M01-613 Va
RGEDVEQSLFLSVREGDSSVINCTYTDSSLTYLYWYKQEPGAGLQLLTYIFSFMDMKQDQRLTVLLNKKDKHLSLRIADTQTGDSAIYFCAGSGGGTDKLIFGTGTRLQVFPN

SEQ ID NO: 137 - protein, 118 aa, synthetic construct
  REGION 1..118: note = A1A2-M01-613 Vb
GAVVSQHPSWVICKSGTSVKIECRSLDFQATTMFWYRQFPKQSLMLMATTDYGSKATYEQGVEKDKFLINHASLTLSTLTVTSAHPEDSSFYICSAREPGQGPWEQYFGPGTRLTVTE

SEQ ID NO: 138 - protein, 269 aa, synthetic construct
  REGION 1..269: note = A1A2-M01-613 a chain
MKTFAGFSFLFLWLQLDCMSRGEDVEQSLFLSVREGDSSVINCTYTDSSLTYLYWYKQEPGAGLQLLTYIFSFMDMKQDQRLTVLLNKKDKHLSLRIADTQTGDSAIYFCAGSGGGTDKLIFGTGTRLQVFPNIQNPEPAVYQLKDPRSQDSTLCLFTDFDSQINVPKTMESGTFITDKCVLDMKAMDSKSNGAIAWSNQTSFTCQDIFKETNATYPSSDVPCDATLTEKSFETDMNLNFQNLLVIVLRILLLKVAGFNLLMTLRLWSS

SEQ ID NO: 139 - protein, 304 aa, synthetic construct
  REGION 1..304: note = A1A2-M01-613 b chain
MLLLLLLLGPGSGLGAVVSQHPSWVICKSGTSVKIECRSLDFQATTMFWYRQFPKQSLMLMATTDYGSKATYEQGVEKDKFLINHASLTLSTLTVTSAHPEDSSFYICSAREPGQGPWEQYFGPGTRLTVTEDLRNVTPPKVSLFEPSKAEIANKQKATLVCLARGFFPDHVELSWWVNGKEVHSGVCTDPQAYKESNYSYCLSSRLRVSATFWHNPRNHFRCQVQFHGLSEEDKWPEGSPKPVTQNISAEAWGRADCGITSASYQQGVLSATILYEILLGKATLYAVLVSTLVVMAMVKRKNS

SEQ ID NO: 140 - protein, 6 aa, synthetic construct
  REGION 1..6: note = A1A2-M01-614 CDR1a
DMLSTY

SEQ ID NO: 141 - protein, 7 aa, synthetic construct
  REGION 1..7: note = A1A2-M01-614 CDR2a
IFIFQAM

SEQ ID NO: 142 - protein, 113 aa, synthetic construct
  REGION 1..113: note = A1A2-M01-614 Va
RGEDVEQSLFLSVREGDSSVINCTYSDMLSTYLYWYKQEPGAGLQLLTYIFIFQAMKQDQRLTVLLNKKDKHLSLRIADTQTGDSAIYFCAGSGGGTDKLIFGTGTRLQVFPN

SEQ ID NO: 143 - protein, 118 aa, synthetic construct
  REGION 1..118: note = A1A2-M01-614 Vb
GAVVSQHPSWVICKSGTSVKIECRSLDFEATTMFWYRQFPKQSLMLMATTDYGSKATYEQGVEKDKFLINHASLTLSTLTVTSAHPEDSSFYICSAREPGQGPWEQYFGPGTRLTVTE

SEQ ID NO: 144 - protein, 269 aa, synthetic construct
  REGION 1..269: note = A1A2-M01-614 a chain
MKTFAGFSFLFLWLQLDCMSRGEDVEQSLFLSVREGDSSVINCTYSDMLSTYLYWYKQEPGAGLQLLTYIFIFQAMKQDQRLTVLLNKKDKHLSLRIADTQTGDSAIYFCAGSGGGTDKLIFGTGTRLQVFPNIQNPEPAVYQLKDPRSQDSTLCLFTDFDSQINVPKTMESGTFITDKCVLDMKAMDSKSNGAIAWSNQTSFTCQDIFKETNATYPSSDVPCDATLTEKSFETDMNLNFQNLLVIVLRILLLKVAGFNLLMTLRLWSS

SEQ ID NO: 145 - protein, 304 aa, synthetic construct
  REGION 1..304: note = A1A2-M01-614 b chain
MLLLLLLLGPGSGLGAVVSQHPSWVICKSGTSVKIECRSLDFEATTMFWYRQFPKQSLMLMATTDYGSKATYEQGVEKDKFLINHASLTLSTLTVTSAHPEDSSFYICSAREPGQGPWEQYFGPGTRLTVTEDLRNVTPPKVSLFEPSKAEIANKQKATLVCLARGFFPDHVELSWWVNGKEVHSGVCTDPQAYKESNYSYCLSSRLRVSATFWHNPRNHFRCQVQFHGLSEEDKWPEGSPKPVTQNISAEAWGRADCGITSASYQQGVLSATILYEILLGKATLYAVLVSTLVVMAMVKRKNS

SEQ ID NO: 146 - protein, 6 aa, synthetic construct
  REGION 1..6: note = A1A2-M01-615 CDR1a
CAFSTY

SEQ ID NO: 147 - protein, 113 aa, synthetic construct
  REGION 1..113: note = A1A2-M01-615 Va
RGEDVEQSLFLSVREGDSSVINCTYICAFSTYLYWYKQEPGAGLQLLTYIFAFESMKQDQRLTVLLNKKDKHLSLRIADTQTGDSAIYFCAGSGGGTDKLIFGTGTRLQVFPN

SEQ ID NO: 148 - protein, 269 aa, synthetic construct
  REGION 1..269: note = A1A2-M01-615 a chain
MKTFAGFSFLFLWLQLDCMSRGEDVEQSLFLSVREGDSSVINCTYICAFSTYLYWYKQEPGAGLQLLTYIFAFESMKQDQRLTVLLNKKDKHLSLRIADTQTGDSAIYFCAGSGGGTDKLIFGTGTRLQVFPNIQNPEPAVYQLKDPRSQDSTLCLFTDFDSQINVPKTMESGTFITDKCVLDMKAMDSKSNGAIAWSNQTSFTCQDIFKETNATYPSSDVPCDATLTEKSFETDMNLNFQNLLVIVLRILLLKVAGFNLLMTLRLWSS

SEQ ID NO: 149 - protein, 7 aa, synthetic construct
  REGION 1..7: note = A1A2-M01-616 CDR2a
IFAFMQM

SEQ ID NO: 150 - protein, 113 aa, synthetic construct
  REGION 1..113: note = A1A2-M01-616 Va
RGEDVEQSLFLSVREGDSSVINCTYTDSSQTYLYWYKQEPGAGLQLLTYIFAFMQMKQDQRLTVLLNKKDKHLSLRIADTQTGDSAIYFCAGSGGGTDKLIFGTGTRLQVFPN

SEQ ID NO: 151 - protein, 269 aa, synthetic construct
  REGION 1..269: note = A1A2-M01-616 a chain
MKTFAGFSFLFLWLQLDCMSRGEDVEQSLFLSVREGDSSVINCTYTDSSQTYLYWYKQEPGAGLQLLTYIFAFMQMKQDQRLTVLLNKKDKHLSLRIADTQTGDSAIYFCAGSGGGTDKLIFGTGTRLQVFPNIQNPEPAVYQLKDPRSQDSTLCLFTDFDSQINVPKTMESGTFITDKCVLDMKAMDSKSNGAIAWSNQTSFTCQDIFKETNATYPSSDVPCDATLTEKSFETDMNLNFQNLLVIVLRILLLKVAGFNLLMTLRLWSS

SEQ ID NO: 152 - protein, 6 aa, synthetic construct
  REGION 1..6: note = A1A2-M01-617 CDR1a
DMFSTY

SEQ ID NO: 153 - protein, 7 aa, synthetic construct
  REGION 1..7: note = A1A2-M01-617 CDR2b
SNEGDQA

SEQ ID NO: 154 - protein, 113 aa, synthetic construct
  REGION 1..113: note = A1A2-M01-617 Va
RGEDVEQSLFLSVREGDSSVINCTYPDMFSTYLYWYKQEPGAGLQLLTYIFAFMQMKQDQRLTVLLNKKDKHLSLRIADTQTGDSAIYFCAGSGGGTDKLIFGTGTRLQVFPN

SEQ ID NO: 155 - protein, 118 aa, synthetic construct
  REGION 1..118: note = A1A2-M01-617 Vb
GAVVSQHPSWVICKSGTSVKIECRSLDFEATTMFWYRQFPKQSLMLMATSNEGDQATYEQGVEKDKFLINHASLTLSTLTVTSAHPEDSSFYICSAREPGQGPWEQYFGPGTRLTVTE

SEQ ID NO: 156 - protein, 269 aa, synthetic construct
  REGION 1..269: note = A1A2-M01-617 a chain
MKTFAGFSFLFLWLQLDCMSRGEDVEQSLFLSVREGDSSVINCTYPDMFSTYLYWYKQEPGAGLQLLTYIFAFMQMKQDQRLTVLLNKKDKHLSLRIADTQTGDSAIYFCAGSGGGTDKLIFGTGTRLQVFPNIQNPEPAVYQLKDPRSQDSTLCLFTDFDSQINVPKTMESGTFITDKCVLDMKAMDSKSNGAIAWSNQTSFTCQDIFKETNATYPSSDVPCDATLTEKSFETDMNLNFQNLLVIVLRILLLKVAGFNLLMTLRLWSS

SEQ ID NO: 157 - protein, 304 aa, synthetic construct
  REGION 1..304: note = A1A2-M01-617 b chain
MLLLLLLLGPGSGLGAVVSQHPSWVICKSGTSVKIECRSLDFEATTMFWYRQFPKQSLMLMATSNEGDQATYEQGVEKDKFLINHASLTLSTLTVTSAHPEDSSFYICSAREPGQGPWEQYFGPGTRLTVTEDLRNVTPPKVSLFEPSKAEIANKQKATLVCLARGFFPDHVELSWWVNGKEVHSGVCTDPQAYKESNYSYCLSSRLRVSATFWHNPRNHFRCQVQFHGLSEEDKWPEGSPKPVTQNISAEAWGRADCGITSASYQQGVLSATILYEILLGKATLYAVLVSTLVVMAMVKRKNS

SEQ ID NO: 158 - protein, 113 aa, synthetic construct
  REGION 1..113: note = A1A2-M01-619 Va
RGEDVEQSLFLSVREGDSSVINCTYTDSSMTYLYWYKQEPGAGLQLLTYIFSFMDMKQDQRLTVLLNKKDKHLSLRIADTQTGDSAIYFCAGSGGGTDKLIFGTGTRLQVFPN

SEQ ID NO: 159 - protein, 118 aa, synthetic construct
  REGION 1..118: note = A1A2-M01-619 Vb
GAVVSQHPSWVICKSGTSVKIECRSLDFEATTMFWYRQFPKQSLMLMATTDYGSKATYEQGVEKDKFLINHASLTLSTLTVTSAHPEDSSFYICSAREPGQGPYEQYFGPGTRLTVTE

SEQ ID NO: 160 - protein, 269 aa, synthetic construct
  REGION 1..269: note = A1A2-M01-619 a chain
MKTFAGFSFLFLWLQLDCMSRGEDVEQSLFLSVREGDSSVINCTYTDSSMTYLYWYKQEPGAGLQLLTYIFSFMDMKQDQRLTVLLNKKDKHLSLRIADTQTGDSAIYFCAGSGGGTDKLIFGTGTRLQVFPNIQNPEPAVYQLKDPRSQDSTLCLFTDFDSQINVPKTMESGTFITDKCVLDMKAMDSKSNGAIAWSNQTSFTCQDIFKETNATYPSSDVPCDATLTEKSFETDMNLNFQNLLVIVLRILLLKVAGFNLLMTLRLWSS

SEQ ID NO: 161 - protein, 304 aa, synthetic construct
  REGION 1..304: note = A1A2-M01-619 b chain
MLLLLLLLGPGSGLGAVVSQHPSWVICKSGTSVKIECRSLDFEATTMFWYRQFPKQSLMLMATTDYGSKATYEQGVEKDKFLINHASLTLSTLTVTSAHPEDSSFYICSAREPGQGPYEQYFGPGTRLTVTEDLRNVTPPKVSLFEPSKAEIANKQKATLVCLARGFFPDHVELSWWVNGKEVHSGVCTDPQAYKESNYSYCLSSRLRVSATFWHNPRNHFRCQVQFHGLSEEDKWPEGSPKPVTQNISAEAWGRADCGITSASYQQGVLSATILYEILLGKATLYAVLVSTLVVMAMVKRKNS

SEQ ID NO: 162 - protein, 13 aa, synthetic construct
  REGION 1..13: note = A1A2-M01-620 CDR3b
SAREPGQAWSDQY

SEQ ID NO: 163 - protein, 118 aa, synthetic construct
  REGION 1..118: note = A1A2-M01-620 Vb
GAVVSQHPSWVICKSGTSVKIECRSLDFEATTMFWYRQFPKQSLMLMATTDYGSKATYEQGVEKDKFLINHASLTLSTLTVTSAHPEDSSFYICSAREPGQAWSDQYFGPGTRLTVTE

SEQ ID NO: 164 - protein, 304 aa, synthetic construct
  REGION 1..304: note = A1A2-M01-620 b chain
MLLLLLLLGPGSGLGAVVSQHPSWVICKSGTSVKIECRSLDFEATTMFWYRQFPKQSLMLMATTDYGSKATYEQGVEKDKFLINHASLTLSTLTVTSAHPEDSSFYICSAREPGQAWSDQYFGPGTRLTVTEDLRNVTPPKVSLFEPSKAEIANKQKATLVCLARGFFPDHVELSWWVNGKEVHSGVCTDPQAYKESNYSYCLSSRLRVSATFWHNPRNHFRCQVQFHGLSEEDKWPEGSPKPVTQNISAEAWGRADCGITSASYQQGVLSATILYEILLGKATLYAVLVSTLVVMAMVKRKNS

SEQ ID NO: 165 - protein, 6 aa, synthetic construct
  REGION 1..6: note = A1A2-M01-621 CDR1a
DSEFTY

SEQ ID NO: 166 - protein, 113 aa, synthetic construct
  REGION 1..113: note = A1A2-M01-621 Va
RGEDVEQSLFLSVREGDSSVINCTYTDSEFTYLYWYKQEPGAGLQLLTYIFAFESMKQDQRLTVLLNKKDKHLSLRIADTQTGDSAIYFCAGSGGGTDKLIFGTGTRLQVFPN

SEQ ID NO: 167 - protein, 269 aa, synthetic construct
  REGION 1..269: note = A1A2-M01-621 a chain
MKTFAGFSFLFLWLQLDCMSRGEDVEQSLFLSVREGDSSVINCTYTDSEFTYLYWYKQEPGAGLQLLTYIFAFESMKQDQRLTVLLNKKDKHLSLRIADTQTGDSAIYFCAGSGGGTDKLIFGTGTRLQVFPNIQNPEPAVYQLKDPRSQDSTLCLFTDFDSQINVPKTMESGTFITDKCVLDMKAMDSKSNGAIAWSNQTSFTCQDIFKETNATYPSSDVPCDATLTEKSFETDMNLNFQNLLVIVLRILLLKVAGFNLLMTLRLWSS

SEQ ID NO: 168 - protein, 113 aa, synthetic construct
  REGION 1..113: note = A1A2-M01-623 Va
RGEDVEQSLFLSVREGDSSVINCTYTDSSQTYLYWYKQEPGAGLQLLTYIFIFQAMKQDQRLTVLLNKKDKHLSLRIADTQTGDSAIYFCAGSGGGTDKLIFGTGTRLQVFPN

SEQ ID NO: 169 - protein, 269 aa, synthetic construct
  REGION 1..269: note = A1A2-M01-623 a chain
MKTFAGFSFLFLWLQLDCMSRGEDVEQSLFLSVREGDSSVINCTYTDSSQTYLYWYKQEPGAGLQLLTYIFIFQAMKQDQRLTVLLNKKDKHLSLRIADTQTGDSAIYFCAGSGGGTDKLIFGTGTRLQVFPNIQNPEPAVYQLKDPRSQDSTLCLFTDFDSQINVPKTMESGTFITDKCVLDMKAMDSKSNGAIAWSNQTSFTCQDIFKETNATYPSSDVPCDATLTEKSFETDMNLNFQNLLVIVLRILLLKVAGFNLLMTLRLWSS

SEQ ID NO: 170 - protein, 6 aa, synthetic construct
  REGION 1..6: note = A1A2-M01-624 CDR1a
YGMSTY

SEQ ID NO: 171 - protein, 113 aa, synthetic construct
  REGION 1..113: note = A1A2-M01-624 Va
RGEDVEQSLFLSVREGDSSVINCTYQYGMSTYLYWYKQEPGAGLQLLTYIFSFMDMKQDQRLTVLLNKKDKHLSLRIADTQTGDSAIYFCAGSGGGTDKLIFGTGTRLQVFPN

SEQ ID NO: 172 - protein, 269 aa, synthetic construct
  REGION 1..269: note = A1A2-M01-624 a chain
MKTFAGFSFLFLWLQLDCMSRGEDVEQSLFLSVREGDSSVINCTYQYGMSTYLYWYKQEPGAGLQLLTYIFSFMDMKQDQRLTVLLNKKDKHLSLRIADTQTGDSAIYFCAGSGGGTDKLIFGTGTRLQVFPNIQNPEPAVYQLKDPRSQDSTLCLFTDFDSQINVPKTMESGTFITDKCVLDMKAMDSKSNGAIAWSNQTSFTCQDIFKETNATYPSSDVPCDATLTEKSFETDMNLNFQNLLVIVLRILLLKVAGFNLLMTLRLWSS

SEQ ID NO: 173 - protein, 113 aa, synthetic construct
  REGION 1..113: note = A1A2-M01-625 Va
RGEDVEQSLFLSVREGDSSVINCTYTDSSMTYLYWYKQEPGAGLQLLTYIFAFESMKQDQRLTVLLNKKDKHLSLRIADTQTGDSAIYFCAGSGGGTDKLIFGTGTRLQVFPN

SEQ ID NO: 174 - protein, 269 aa, synthetic construct
  REGION 1..269: note = A1A2-M01-625 a chain
MKTFAGFSFLFLWLQLDCMSRGEDVEQSLFLSVREGDSSVINCTYTDSSMTYLYWYKQEPGAGLQLLTYIFAFESMKQDQRLTVLLNKKDKHLSLRIADTQTGDSAIYFCAGSGGGTDKLIFGTGTRLQVFPNIQNPEPAVYQLKDPRSQDSTLCLFTDFDSQINVPKTMESGTFITDKCVLDMKAMDSKSNGAIAWSNQTSFTCQDIFKETNATYPSSDVPCDATLTEKSFETDMNLNFQNLLVIVLRILLLKVAGFNLLMTLRLWSS

SEQ ID NO: 175 - protein, 118 aa, synthetic construct
  REGION 1..118: note = A1A2-M01-626 Vb
GAVVSQHPSWVICKSGTSVKIECRSLDFPIERMFWYRQFPKQSLMLMATTDYGSKATYEQGVEKDKFLINHASLTLSTLTVTSAHPEDSSFYICSAREPGQGPFEQYFGPGTRLTVTE

SEQ ID NO: 176 - protein, 304 aa, synthetic construct
  REGION 1..304: note = A1A2-M01-626 b chain
MLLLLLLLGPGSGLGAVVSQHPSWVICKSGTSVKIECRSLDFPIERMFWYRQFPKQSLMLMATTDYGSKATYEQGVEKDKFLINHASLTLSTLTVTSAHPEDSSFYICSAREPGQGPFEQYFGPGTRLTVTEDLRNVTPPKVSLFEPSKAEIANKQKATLVCLARGFFPDHVELSWWVNGKEVHSGVCTDPQAYKESNYSYCLSSRLRVSATFWHNPRNHFRCQVQFHGLSEEDKWPEGSPKPVTQNISAEAWGRADCGITSASYQQGVLSATILYEILLGKATLYAVLVSTLVVMAMVKRKNS

SEQ ID NO: 177 - protein, 9 aa, synthetic construct
  REGION 1..9: note = gp100 target antigen peptide
YLEPGPVTV